European Patent Specification EP 3 461 486 B1, published October 25, 2023. Title: A pharmaceutical composition for the prevention or treatment of dementia and improvement of cognitive function comprising extract of Salicornia spp. Applicant: PHYTO CORPORATION INC. The sequence listing filed with the application follows.

SEQUENCE LISTING (12 sequences)

SEQ ID NO: 1 - DNA, 20 bp, Artificial Sequence
  iNOS-F
tgaagaaaaccccttgtgct

SEQ ID NO: 2 - DNA, 20 bp, Artificial Sequence
  iNOS-R
ttctgtgctgtcccagtgag

SEQ ID NO: 3 - DNA, 22 bp, Artificial Sequence
  COX2-F
caagacagatcataagcgagga

SEQ ID NO: 4 - DNA, 21 bp, Artificial Sequence
  COX2-R
ggcgcagtttatgttgtctgt

SEQ ID NO: 5 - DNA, 21 bp, Artificial Sequence
  TNFa-F
ccaccacgctcttctgtctac

SEQ ID NO: 6 - DNA, 20 bp, Artificial Sequence
  TNFa-R
agggtctgggccatagaact

SEQ ID NO: 7 - DNA, 20 bp, Artificial Sequence
  IL-1b-F
tgtgaaatgccaccttttga

SEQ ID NO: 8 - DNA, 20 bp, Artificial Sequence
  IL-1b-R
ggtcaaaggtttggaagcag

SEQ ID NO: 9 - DNA, 20 bp, Artificial Sequence
  IL-6-F
tgatgcacttgcagaaaaca

SEQ ID NO: 10 - DNA, 23 bp, Artificial Sequence
  IL-6-R
accagaggaaattttcaataggc

SEQ ID NO: 11 - DNA, 20 bp, Artificial Sequence
  GAPDH-F
aagggctcatgaccacagtc

SEQ ID NO: 12 - DNA, 20 bp, Artificial Sequence
  GAPDH-R
ttcagctctgggatgacctt